European Patent Application EP 4 245 843 A1, published September 20, 2023. Title: Carotenoid compounds. Applicant: Ezaki Glico Co., Ltd. The sequence listing filed with the application follows.

SEQUENCE LISTING (12 sequences)

SEQ ID NO: 1 - DNA, 321 bp, human
atggattctagctcaaactattgtaatcaaatgatgaaatcccgtaacctgaccaaagaccgctgtaaacctgtcaatacctttgtccacgaatctttagccgatgttcaagccgtgtgttctcaaaaaaatgtagcctgtaaaaatggccaaaccaactgttatcaatcatattccaccatgtccattaccgattgtcgcgaaacaggatcttccaaatatccaaattgtgcatataaaactacccaagcgaacaaacatattatcgtagcatgtgaaggcaacccgtacgtacctgtccacttcgacgcatcagtgtaa

SEQ ID NO: 2 - protein, 106 aa, human
MDSSSNYCNQMMKSRNLTKDRCKPVNTFVHESLADVQAVCSQKNVACKNGQTNCYQSYSTMSITDCRETGSSKYPNCAYKTTQANKHIIVACEGNPYVPVHFDASV

SEQ ID NO: 3 - DNA, 60 bp, Artificial Sequence
  S-Tag coding oligonucloetide with substitution at 34th to 36th position by phenylalanine coding sequence
aaagaaaccgctgctgcgaaatttgaacgccagttcatggactcgtctactagcgcagct

SEQ ID NO: 4 - protein, 20 aa, Artificial Sequence
  S-Tag amino sequence with substitution at 12th position by phenylalanine
KETAAAKFERQFMDSSTSAA

SEQ ID NO: 5 - DNA, 1446 bp, Artificial Sequence
  S-Tag introduced CaCCS
atggcaaaagaaaccgctgctgcgaaatttgaacgccagttcatggactcgtctactagcgcagctatgtttcattatcgtaacaaaagcagcacccatttttgcagctttctggatctggcgccgaccagcaaaccggaaagcctggatgtgaatatcagctgggttgataccgatctggatggcgccgaatttgatgtgattatcattggtaccggtccggccggcctgcgtctggcagaacaggttagcaaatatggtattaaagtgtgctgtgttgatccgagcccgctgagcatgtggccgaacaattatggcgtgtgggttgatgaatttgaaaaactgggtctggaagattgcctggatcataaatggccggtgagctgtgttcatatcagcgatcataaaaccaaatatctggatcgcccgtatggtcgcgtgagccgtaaaaaactgaaactgaaactgctgaacagctgcgtggaaaaccgtgttaaattctacaaagcgaaagtgctgaaagttaaacatgaagaatttgaaagcagcattgtgtgtgatgatggccgcaaaatcagcggtagcctgattgttgatgcgagcggctatgccagcgattttatcgaatatgataaaccgcgtaatcatggctatcaggtggcgcatggtattctggccgaagttgataatcatccgtttgatctggataaaatgatgctgatggattggcgcgatagccatctgggtaacgaaccgtatctgcgtgtgaaaaataccaaagaaccgacctttctgtatgcgatgccgtttgatcgcaatctggtgtttctggaagaaaccagcctggttagccgtccgatgctgagctatatggaagtgaaacgtcgcatggttgcccgcctgcgtcatctgggcattaaagtgcgcagcgttctggaagaagaaaaatgtgtgatcacgatgggcggcccgctgccgcgtattccgcagaacgttatggcgatcggcggtaccagcggcattgtgcatccgagcagcggttatatggttgcgcgcagcatggcgctggcaccggtgctggcggaagccatcgttgaaagcctgggcagcacccgcatgattcgtggtagccagctgtatcatcgcgtgtggaatggtctgtggccgagcgatcgtcgccgtgttcgtgaatgctattgttttggcatggaaaccttattaaaactggatctggaaggtacccgccgtctgtttgatgcgtttttcgatgttgatccgaaatattggcatggctttctgagcagccgcctgagcgtgaaagaactggccgttctgagcctgtacctgtttggtcatgcgagcaacctggcccgtctggatatcgtgaccaaatgtaccgtgccgctggttaaactgctgggcaatctggcgattgaaagcctgtaa

SEQ ID NO: 6 - protein, 481 aa, Artificial Sequence
  S-Tag introduced CaCCS
MAKETAAAKFERQFMDSSTSAAMFHYRNKSSTHFCSFLDLAPTSKPESLDVNISWVDTDLDGAEFDVIIIGTGPAGLRLAEQVSKYGIKVCCVDPSPLSMWPNNYGVWVDEFEKLGLEDCLDHKWPVSCVHISDHKTKYLDRPYGRVSRKKLKLKLLNSCVENRVKFYKAKVLKVKHEEFESSIVCDDGRKISGSLIVDASGYASDFIEYDKPRNHGYQVAHGILAEVDNHPFDLDKMMLMDWRDSHLGNEPYLRVKNTKEPTFLYAMPFDRNLVFLEETSLVSRPMLSYMEVKRRMVARLRHLGIKVRSVLEEEKCVITMGGPLPRIPQNVMAIGGTSGIVHPSSGYMVARSMALAPVLAEAIVESLGSTRMIRGSQLYHRVWNGLWPSDRRRVRECYCFGMETLLKLDLEGTRRLFDAFFDVDPKYWHGFLSSRLSVKELAVLSLYLFGHASNLARLDIVTKCTVPLVKLLGNLAIESL

SEQ ID NO: 7 - DNA, 1506 bp, Artificial Sequence
  S-Tag introduced CaCCS via linker
atgtcgaaagaaaccgctgctgcgaaatttgaacgccagttcatggactcgtctactagtgcagctggttcaggtagtggttcaggttctggttcaggttcaggtagtggttcaggttctggttcaatgtttcattatcgtaacaaaagcagcacccatttttgcagctttctggatctggcgccgaccagcaaaccggaaagcctggatgtgaatatcagctgggttgataccgatctggatggcgccgaatttgatgtgattatcattggtaccggtccggccggcctgcgtctggcagaacaggttagcaaatatggtattaaagtgtgctgtgttgatccgagcccgctgagcatgtggccgaacaattatggcgtgtgggttgatgaatttgaaaaactgggtctggaagattgcctggatcataaatggccggtgagctgtgttcatatcagcgatcataaaaccaaatatctggatcgcccgtatggtcgcgtgagccgtaaaaaactgaaactgaaactgctgaacagctgcgtggaaaaccgtgttaaattctacaaagcgaaagtgctgaaagttaaacatgaagaatttgaaagcagcattgtgtgtgatgatggccgcaaaatcagcggtagcctgattgttgatgcgagcggctatgccagcgattttatcgaatatgataaaccgcgtaatcatggctatcaggtggcgcatggtattctggccgaagttgataatcatccgtttgatctggataaaatgatgctgatggattggcgcgatagccatctgggtaacgaaccgtatctgcgtgtgaaaaataccaaagaaccgacctttctgtatgcgatgccgtttgatcgcaatctggtgtttctggaagaaaccagcctggttagccgtccgatgctgagctatatggaagtgaaacgtcgcatggttgcccgcctgcgtcatctgggcattaaagtgcgcagcgttctggaagaagaaaaatgtgtgatcacgatgggcggcccgctgccgcgtattccgcagaacgttatggcgatcggcggtaccagcggcattgtgcatccgagcagcggttatatggttgcgcgcagcatggcgctggcaccggtgctggcggaagccatcgttgaaagcctgggcagcacccgcatgattcgtggtagccagctgtatcatcgcgtgtggaatggtctgtggccgagcgatcgtcgccgtgttcgtgaatgctattgttttggcatggaaaccttattaaaactggatctggaaggtacccgccgtctgtttgatgcgtttttcgatgttgatccgaaatattggcatggctttctgagcagccgcctgagcgtgaaagaactggccgttctgagcctgtacctgtttggtcatgcgagcaacctggcccgtctggatatcgtgaccaaatgtaccgtgccgctggttaaactgctgggcaatctggcgattgaaagcctgtaa

SEQ ID NO: 8 - protein, 501 aa, Artificial Sequence
  S-Tag introduced CaCCS via linker
MSKETAAAKFERQFMDSSTSAAGSGSGSGSGSGSGSGSGSGSMFHYRNKSSTHFCSFLDLAPTSKPESLDVNISWVDTDLDGAEFDVIIIGTGPAGLRLAEQVSKYGIKVCCVDPSPLSMWPNNYGVWVDEFEKLGLEDCLDHKWPVSCVHISDHKTKYLDRPYGRVSRKKLKLKLLNSCVENRVKFYKAKVLKVKHEEFESSIVCDDGRKISGSLIVDASGYASDFIEYDKPRNHGYQVAHGILAEVDNHPFDLDKMMLMDWRDSHLGNEPYLRVKNTKEPTFLYAMPFDRNLVFLEETSLVSRPMLSYMEVKRRMVARLRHLGIKVRSVLEEEKCVITMGGPLPRIPQNVMAIGGTSGIVHPSSGYMVARSMALAPVLAEAIVESLGSTRMIRGSQLYHRVWNGLWPSDRRRVRECYCFGMETLLKLDLEGTRRLFDAFFDVDPKYWHGFLSSRLSVKELAVLSLYLFGHASNLARLDIVTKCTVPLVKLLGNLAIESL

SEQ ID NO: 9 - DNA, 2073 bp, Artificial Sequence
  S-Tag introduced CaZEP
atgtcgaaagaaaccgctgctgcgaaatttgaacgccagttcatggactcgtctactagtgcagctatgaccatgattacgaattcgatgtatagcaccgtgttttataccagcgttcatccgagcaccagcgtgtttagccgcaaacagctgccgctgctgattagcaaagattttccggccgaactgtatcatagcctgccgtgcaaaagcctggaaaatggtcatattaagaaagtgaaaggcgttaaagccaccctggccgaagcaccggccaccccgaccgaaaaatctaacagcgaagtgccgcagaaaaaactgaaagtgctggttgccggcggtggcattggtggcctggtgtttgcgctggcggcgaaaaagaaaggctttgatgtgctggtttttgaacgtgatctgagcgccatccgcggcgaaggccagtatcgtggcccgattcagatccagagcaatgccctggcggccctggaagcgattgatatggatgtggccgaagaaatcatgaacgcgggttgcattaccggccagcgtatcaatggtctggttgatggtattagcggcaactggtattgtaaatttgatacctttaccccggccgtggaacgcggcctgccggtgacccgtgttattagccgcatgaccctgcagcagatcctggcacgtgccgtgggtgaagatgttattatgaacgaaagcaatgtggttaactttgaagatgatggcgaaaaagtgaccgtggttctggaaaatggtcagcgctttaccggcgatctgctggttggtgccgatggcatccgtagcaaagtgcgcaccaacctgtttggtcatagcgaagcgacctatagcggttatacctgttataccggcattgccgattttgttccggcggatatcgataccgtgggttatcgtgtttttctgggccataaacagtattttgtgagcagcgatgttggtggcggtaaaatgcagtggtatgcgtttcataatgaaccggccggcggtgtggatgccccgaatggcaagaaagaacgcctgctgaaaatttttggcggttggtgcgataatgtgatcgatctgctggttgccaccgatgaagatgcgattctgcgtcgcgatatctatgatcgtccgccgacctttaattggggtcgtggtcgtgtgaccctgctgggtgatagcgttcatgccatgcagccgaacctgggtcagggcggttgtatggccattgaagatagctatcagctggcgctggaactggaaaaagcctggagccgcagcgccgaaagcggtagcccgatggatgttatcagcagcctgcgtagctatgaaagcgcccgtaaactgcgcgtgggtgttattcatggcctggcccgtatggccgcaatcatggcaagcacctataaagcgtatctgggcgtgggtctgggtccgctgagctttctgaccaaatatcgtattccgcacccgggtcgtgttggcggtcgtgtgtttgttgatctgggcatgccgctgatgctgagctgggtgctgggcggtaatggtgataaactggaaggccgtatccagcattgccgcctgagcgaaaaagccaacgatcagctgcgtcgctggtttgaagatgatgatgcgctggaacgcgccaccgatgccgaatggctgctgctgccggccgcaaatggcaatagcgcgctggaaaccattgtgctgagccgtgatgaagatgttccgtgcaccattggtagcgtgagccataccaacatcccgggcaaaagcgtggttctgccgctgccgcaggttagcgaaatgcatgcccagattagctgtaaaaacaatgcgtttttcgtgaccgattttcagagcgaacatggtacctgggttatcgataatgaaggccgtcgctatcgcgtgagcccgaactttccgatgcgttttcatagcagcgatgtgattgtttttggtagcgataaagcggcctttcgcgtgaaaaccatgaaatttccgagcaaaaccgccgaagcgaaagaagaacgtaaagtggttggcaccgcgtaa

SEQ ID NO: 10 - protein, 690 aa, Artificial Sequence
  S-Tag introduced CaZEP
MSKETAAAKFERQFMDSSTSAAMTMITNSMYSTVFYTSVHPSTSVFSRKQLPLLISKDFPAELYHSLPCKSLENGHIKKVKGVKATLAEAPATPTEKSNSEVPQKKLKVLVAGGGIGGLVFALAAKKKGFDVLVFERDLSAIRGEGQYRGPIQIQSNALAALEAIDMDVAEEIMNAGCITGQRINGLVDGISGNWYCKFDTFTPAVERGLPVTRVISRMTLQQILARAVGEDVIMNESNVVNFEDDGEKVTVVLENGQRFTGDLLVGADGIRSKVRTNLFGHSEATYSGYTCYTGIADFVPADIDTVGYRVFLGHKQYFVSSDVGGGKMQWYAFHNEPAGGVDAPNGKKERLLKIFGGWCDNVIDLLVATDEDAILRRDIYDRPPTFNWGRGRVTLLGDSVHAMQPNLGQGGCMAIEDSYQLALELEKAWSRSAESGSPMDVISSLRSYESARKLRVGVIHGLARMAAIMASTYKAYLGVGLGPLSFLTKYRIPHPGRVGGRVFVDLGMPLMLSWVLGGNGDKLEGRIQHCRLSEKANDQLRRWFEDDDALERATDAEWLLLPAANGNSALETIVLSRDEDVPCTIGSVSHTNIPGKSVVLPLPQVSEMHAQISCKNNAFFVTDFQSEHGTWVIDNEGRRYRVSPNFPMRFHSSDVIVFGSDKAAFRVKTMKFPSKTAEAKEERKVVGTA

SEQ ID NO: 11 - DNA, 2133 bp, Artificial Sequence
  S-Tag introduced CaZEP via linker
atgtcgaaagaaaccgctgctgcgaaatttgaacgccagttcatggactcgtctactagtgcagctggttcaggtagtggttcaggttctggttcaggttcaggtagtggttcaggttctggttcaatgaccatgattacgaattcgatgtatagcaccgtgttttataccagcgttcatccgagcaccagcgtgtttagccgcaaacagctgccgctgctgattagcaaagattttccggccgaactgtatcatagcctgccgtgcaaaagcctggaaaatggtcatattaagaaagtgaaaggcgttaaagccaccctggccgaagcaccggccaccccgaccgaaaaatctaacagcgaagtgccgcagaaaaaactgaaagtgctggttgccggcggtggcattggtggcctggtgtttgcgctggcggcgaaaaagaaaggctttgatgtgctggtttttgaacgtgatctgagcgccatccgcggcgaaggccagtatcgtggcccgattcagatccagagcaatgccctggcggccctggaagcgattgatatggatgtggccgaagaaatcatgaacgcgggttgcattaccggccagcgtatcaatggtctggttgatggtattagcggcaactggtattgtaaatttgatacctttaccccggccgtggaacgcggcctgccggtgacccgtgttattagccgcatgaccctgcagcagatcctggcacgtgccgtgggtgaagatgttattatgaacgaaagcaatgtggttaactttgaagatgatggcgaaaaagtgaccgtggttctggaaaatggtcagcgctttaccggcgatctgctggttggtgccgatggcatccgtagcaaagtgcgcaccaacctgtttggtcatagcgaagcgacctatagcggttatacctgttataccggcattgccgattttgttccggcggatatcgataccgtgggttatcgtgtttttctgggccataaacagtattttgtgagcagcgatgttggtggcggtaaaatgcagtggtatgcgtttcataatgaaccggccggcggtgtggatgccccgaatggcaagaaagaacgcctgctgaaaatttttggcggttggtgcgataatgtgatcgatctgctggttgccaccgatgaagatgcgattctgcgtcgcgatatctatgatcgtccgccgacctttaattggggtcgtggtcgtgtgaccctgctgggtgatagcgttcatgccatgcagccgaacctgggtcagggcggttgtatggccattgaagatagctatcagctggcgctggaactggaaaaagcctggagccgcagcgccgaaagcggtagcccgatggatgttatcagcagcctgcgtagctatgaaagcgcccgtaaactgcgcgtgggtgttattcatggcctggcccgtatggccgcaatcatggcaagcacctataaagcgtatctgggcgtgggtctgggtccgctgagctttctgaccaaatatcgtattccgcacccgggtcgtgttggcggtcgtgtgtttgttgatctgggcatgccgctgatgctgagctgggtgctgggcggtaatggtgataaactggaaggccgtatccagcattgccgcctgagcgaaaaagccaacgatcagctgcgtcgctggtttgaagatgatgatgcgctggaacgcgccaccgatgccgaatggctgctgctgccggccgcaaatggcaatagcgcgctggaaaccattgtgctgagccgtgatgaagatgttccgtgcaccattggtagcgtgagccataccaacatcccgggcaaaagcgtggttctgccgctgccgcaggttagcgaaatgcatgcccagattagctgtaaaaacaatgcgtttttcgtgaccgattttcagagcgaacatggtacctgggttatcgataatgaaggccgtcgctatcgcgtgagcccgaactttccgatgcgttttcatagcagcgatgtgattgtttttggtagcgataaagcggcctttcgcgtgaaaaccatgaaatttccgagcaaaaccgccgaagcgaaagaagaacgtaaagtggttggcaccgcgtaa

SEQ ID NO: 12 - protein, 710 aa, Artificial Sequence
  S-Tag introduced CaZEP via linker
MSKETAAAKFERQFMDSSTSAAGSGSGSGSGSGSGSGSGSGSMTMITNSMYSTVFYTSVHPSTSVFSRKQLPLLISKDFPAELYHSLPCKSLENGHIKKVKGVKATLAEAPATPTEKSNSEVPQKKLKVLVAGGGIGGLVFALAAKKKGFDVLVFERDLSAIRGEGQYRGPIQIQSNALAALEAIDMDVAEEIMNAGCITGQRINGLVDGISGNWYCKFDTFTPAVERGLPVTRVISRMTLQQILARAVGEDVIMNESNVVNFEDDGEKVTVVLENGQRFTGDLLVGADGIRSKVRTNLFGHSEATYSGYTCYTGIADFVPADIDTVGYRVFLGHKQYFVSSDVGGGKMQWYAFHNEPAGGVDAPNGKKERLLKIFGGWCDNVIDLLVATDEDAILRRDIYDRPPTFNWGRGRVTLLGDSVHAMQPNLGQGGCMAIEDSYQLALELEKAWSRSAESGSPMDVISSLRSYESARKLRVGVIHGLARMAAIMASTYKAYLGVGLGPLSFLTKYRIPHPGRVGGRVFVDLGMPLMLSWVLGGNGDKLEGRIQHCRLSEKANDQLRRWFEDDDALERATDAEWLLLPAANGNSALETIVLSRDEDVPCTIGSVSHTNIPGKSVVLPLPQVSEMHAQISCKNNAFFVTDFQSEHGTWVIDNEGRRYRVSPNFPMRFHSSDVIVFGSDKAAFRVKTMKFPSKTAEAKEERKVVGTA